European Patent Application EP 4 368 719 A1, published May 15, 2024. Title: Transposon system and its use. Applicant: NeogenTC Corp. The sequence listing filed with the application follows.

SEQUENCE LISTING (30 sequences)

SEQ ID NO: 1 - DNA, 157 bp, synthetic construct
  source 1..157: mol_type = other DNA
ttaacacttggattgcgggaaacgagttaagtcggctcgcgtgaattgcgcgtactccgcgggagccgtcttaactcggttcatatagatttgcggtggagtgcgggaaacgtgtaaactcgggccgattgtaactgcgtattaccaaatatttgtt

SEQ ID NO: 2 - DNA, 212 bp, synthetic construct
  source 1..212: mol_type = other DNA
aattatttatgtactgaatagataaaaaaatgtctgtgattgaataaattttcattttttacacaagaaaccgaaaatttcatttcaatcgaacccatacttcaaaagatataggcattttaaactaactctgattttgcgcgggaaacctaaataattgcccgcgccatcttatattttggcgggaaattcacccgacaccgtagtgttaa

SEQ ID NO: 3 - DNA, 13 bp, synthetic construct
  source 1..13: mol_type = other DNA
ttaacacttggat

SEQ ID NO: 4 - DNA, 33 bp, synthetic construct
  source 1..33: mol_type = other DNA
ttaacacttggattgcgggaaacgagttaagtc

SEQ ID NO: 5 - DNA, 71 bp, synthetic construct
  source 1..71: mol_type = other DNA
ttaacacttggattgcgggaaacgagttaagtcggctcgcgtgaattgcgcgtactccgcgggagccgtct

SEQ ID NO: 6 - DNA, 110 bp, synthetic construct
  source 1..110: mol_type = other DNA
ttaacacttggattgcgggaaacgagttaagtcggctcgcgtgaattgcgcgtactccgcgggagccgtcttaactcggttcatatagatttgcggtggagtgcgggaaa

SEQ ID NO: 7 - DNA, 26 bp, synthetic construct
  source 1..26: mol_type = other DNA
ttaacacttggattgcgggaaacgag

SEQ ID NO: 8 - DNA, 15 bp, synthetic construct
  source 1..15: mol_type = other DNA
tgcgggaaacgagtt

SEQ ID NO: 9 - DNA, 66 bp, synthetic construct
  source 1..66: mol_type = other DNA
aacctaaataattgcccgcgccatcttatattttggcgggaaattcacccgacaccgtagtgttaa

SEQ ID NO: 10 - DNA, 91 bp, synthetic construct
  source 1..91: mol_type = other DNA
aaactaactctgattttgcgcgggaaacctaaataattgcccgcgccatcttatattttggcgggaaattcacccgacaccgtagtgttaa

SEQ ID NO: 11 - DNA, 151 bp, synthetic construct
  source 1..151: mol_type = other DNA
cacaagaaaccgaaaatttcatttcaatcgaacccatacttcaaaagatataggcattttaaactaactctgattttgcgcgggaaacctaaataattgcccgcgccatcttatattttggcgggaaattcacccgacaccgtagtgttaa

SEQ ID NO: 12 - DNA, 37 bp, synthetic construct
  source 1..37: mol_type = other DNA
attttggcgggaaattcacccgacaccgtagtgttaa

SEQ ID NO: 13 - DNA, 30 bp, synthetic construct
  source 1..30: mol_type = other DNA
ttggcgggaaattcacccgacaccgtagtg

SEQ ID NO: 14 - DNA, 18 bp, synthetic construct
  source 1..18: mol_type = other DNA
aactctgattttgcgcgg

SEQ ID NO: 15 - DNA, 66 bp, synthetic construct
  source 1..66: mol_type = other DNA
ttaacactacggtgtcgggtgaatttcccgccaaaatataagatggcgcgggcaattatttaggtt

SEQ ID NO: 16 - DNA, 91 bp, synthetic construct
  source 1..91: mol_type = other DNA
ttaacactacggtgtcgggtgaatttcccgccaaaatataagatggcgcgggcaattatttaggtttcccgcgcaaaatcagagttagttt

SEQ ID NO: 17 - DNA, 152 bp, synthetic construct
  source 1..152: mol_type = other DNA
ttaacactacggtgtcgggtgaatttcccgccaaaatataagatggcgcgggcaattatttaggtttcccgcgcaaaatcagagttagtttaaaatgcctatatcttttgaagtatgggttcgattgaaatgaaattttcggtttcttgtgt

SEQ ID NO: 18 - protein, 572 aa, synthetic construct
MSQHSDYSDDEFCADKLSNYSCDSDLENASTSDEDSSDDEVMVRPRTLRRRRISSSSSDSESDIEGGREEWSHVDNPPVLEDFLGHQGLNTDAVINNIEDAVKLFIGDDFFEFLVEESNRYYNQNRNNFKLSKKSLKWKDITPQEMKKFLGLIVLMGQVRKDRRDDYWTTEPWTETPYFGKTMTRDRFRQIWKAWHFNNNADIVNESDRLCKVRPVLDYFVPKFINIYKPHQQLSLDEGIVPWRGRLFFRVYNAGKIVKYGILVRLLCESDTGYICNMEIYCGEGKRLLETIQTVVSPYTDSWYHIYMDNYYNSVANCEALMKNKFRICGTIRKNRGIPKDFQTISLKKGETKFIRKNDILLQVWQSKKPVYLISSIHSAEMEESQNIDRTSKKKIVKPNALIDYNKHMKGVDRADQYLSYYSILRRTVKWTKRLAMYMINCALFNSYAVYKSVRQRKMGFKMFLKQTAIHWLTDDIPEDMDIVPDLQPVPSTSGMRAKPPTSDPPCRLSMDMRKHTLQAIVGSGKKKNILRRCRVCSVHKLRSETRYMCKFCNIPLHKGACFEKYHTLKNY

SEQ ID NO: 19 - DNA, 1716 bp, synthetic construct
  source 1..1716: mol_type = other DNA
atgtcgcaacactcagattactccgacgatgaattttgtgctgacaaactgtccaattattcatgcgatagcgacctcgaaaacgcttccacgtctgatgaagatagcagcgatgatgaagtaatggtgaggcctcgcaccctccgccgtcgccgcatcagctcttcgagctctgattctgaatccgatattgagggtggccgcgaggagtggtcccacgtagacaatccgccggtgctggaggacttcctaggccaccaaggtctgaacactgacgcagtaatcaacaatatcgaagatgcagttaaactgtttatcggtgacgatttcttcgagtttctggtggaggaatctaaccggtactataaccagaatcgtaataacttcaagctctctaaaaagtctctgaagtggaaggacatcacccctcaggagatgaaaaagttcctcggtctgatcgttctgatgggccaagttcgcaaggatcgtcgtgacgactattggactaccgaaccgtggacggaaactccatactttggcaagaccatgactcgtgaccgtttccgtcagatctggaaggcctggcacttcaataacaacgctgacattgtcaacgagtctgatcgtctgtgtaaggttcgccctgtgctggattacttcgttccaaaattcattaacatttacaaaccacatcagcagctgtccctggatgagggcatcgtgccgtggcgcggccgcctgttcttccgtgtctataatgctggcaagattgtgaagtacggtatcctggttcgcctgctgtgcgaaagcgacactggctacatctgtaacatggagatctactgcggcgagggcaaacgtctcctcgaaactatccagaccgtcgtgtctccatacacggattcctggtatcatatttacatggataactattataacagcgtggctaactgtgaagctctgatgaaaaataagttccgtatttgcggtactatccgtaagaatcgtggaattccgaaagatttccagaccatctccctgaaaaagggtgaaactaagttcattcgcaaaaacgacatcctcctgcaagtctggcagtctaaaaagcctgtatatctgatctcatctattcacagcgctgaaatggaagaatctcagaacattgatcgcacctccaagaaaaagatcgtcaaaccgaatgcattgattgattacaacaagcacatgaagggcgttgatcgtgctgaccagtacctgtcttattactctatcctgcgccgtactgtgaagtggactaaacgtctcgctatgtacatgattaattgtgcgctgttcaattcttacgctgtgtataaaagcgtgcgtcagcgcaaaatgggctttaaaatgttcctgaagcagacggctattcactggctgaccgacgatattccggaagatatggacattgtcccggatctccagccggtaccgagcaccagcggtatgcgtgctaaacctccgactagtgatccgccttgccgtctgtctatggatatgcgtaagcataccctgcaggcaattgtgggctctggcaaaaagaaaaatatcctgcgtcgttgccgcgtatgctctgtacacaaactgcgttctgagactcgttatatgtgtaaattttgcaatattccactccacaagggtgcgtgcttcgagaagtaccatacgctgaagaactat

SEQ ID NO: 20 - RNA, 1716 nt, synthetic construct
  source 1..1716: mol_type = other RNA
atgtcgcaacactcagattactccgacgatgaattttgtgctgacaaactgtccaattattcatgcgatagcgacctcgaaaacgcttccacgtctgatgaagatagcagcgatgatgaagtaatggtgaggcctcgcaccctccgccgtcgccgcatcagctcttcgagctctgattctgaatccgatattgagggtggccgcgaggagtggtcccacgtagacaatccgccggtgctggaggacttcctaggccaccaaggtctgaacactgacgcagtaatcaacaatatcgaagatgcagttaaactgtttatcggtgacgatttcttcgagtttctggtggaggaatctaaccggtactataaccagaatcgtaataacttcaagctctctaaaaagtctctgaagtggaaggacatcacccctcaggagatgaaaaagttcctcggtctgatcgttctgatgggccaagttcgcaaggatcgtcgtgacgactattggactaccgaaccgtggacggaaactccatactttggcaagaccatgactcgtgaccgtttccgtcagatctggaaggcctggcacttcaataacaacgctgacattgtcaacgagtctgatcgtctgtgtaaggttcgccctgtgctggattacttcgttccaaaattcattaacatttacaaaccacatcagcagctgtccctggatgagggcatcgtgccgtggcgcggccgcctgttcttccgtgtctataatgctggcaagattgtgaagtacggtatcctggttcgcctgctgtgcgaaagcgacactggctacatctgtaacatggagatctactgcggcgagggcaaacgtctcctcgaaactatccagaccgtcgtgtctccatacacggattcctggtatcatatttacatggataactattataacagcgtggctaactgtgaagctctgatgaaaaataagttccgtatttgcggtactatccgtaagaatcgtggaattccgaaagatttccagaccatctccctgaaaaagggtgaaactaagttcattcgcaaaaacgacatcctcctgcaagtctggcagtctaaaaagcctgtatatctgatctcatctattcacagcgctgaaatggaagaatctcagaacattgatcgcacctccaagaaaaagatcgtcaaaccgaatgcattgattgattacaacaagcacatgaagggcgttgatcgtgctgaccagtacctgtcttattactctatcctgcgccgtactgtgaagtggactaaacgtctcgctatgtacatgattaattgtgcgctgttcaattcttacgctgtgtataaaagcgtgcgtcagcgcaaaatgggctttaaaatgttcctgaagcagacggctattcactggctgaccgacgatattccggaagatatggacattgtcccggatctccagccggtaccgagcaccagcggtatgcgtgctaaacctccgactagtgatccgccttgccgtctgtctatggatatgcgtaagcataccctgcaggcaattgtgggctctggcaaaaagaaaaatatcctgcgtcgttgccgcgtatgctctgtacacaaactgcgttctgagactcgttatatgtgtaaattttgcaatattccactccacaagggtgcgtgcttcgagaagtaccatacgctgaagaactat

SEQ ID NO: 21 - DNA, 48 bp, synthetic construct
  source 1..48: mol_type = other DNA
gatcccactagtgtcgacaccagtctctaattttttttttcaaaaaaa

SEQ ID NO: 22 - DNA, 61 bp, synthetic construct
  source 1..61: mol_type = other DNA
cgaagagtaaccgttgctaggagagaccgtggctgaatgagactggtgtcgacactagtgg

SEQ ID NO: 23 - DNA, 28 bp, synthetic construct
  source 1..28: mol_type = other DNA
cgaagagtaaccgttgctaggagagacc

SEQ ID NO: 24 - DNA, 24 bp, synthetic construct
  source 1..24: mol_type = other DNA
ccctatagtgagtcgtattaccaa

SEQ ID NO: 25 - DNA, 26 bp, synthetic construct
  source 1..26: mol_type = other DNA
cattaccctgttatccctagctagca

SEQ ID NO: 26 - DNA, 28 bp, synthetic construct
  source 1..28: mol_type = other DNA
cgaagagtaaccgttgctaggagagacc

SEQ ID NO: 27 - DNA, 25 bp, synthetic construct
  source 1..25: mol_type = other DNA
gtggctgaatgagactggtgtcgac

SEQ ID NO: 28 - DNA, 20 bp, synthetic construct
  source 1..20: mol_type = other DNA
ggtcatagctgtttcctgct

SEQ ID NO: 29 - DNA, 27 bp, synthetic construct
  source 1..27: mol_type = other DNA
catttcaatcgaacccatacttcaaaa

SEQ ID NO: 30 - DNA, 25 bp, synthetic construct
  source 1..25: mol_type = other DNA
gtggctgaatgagactggtgtcgac